European Patent Application EP 4 316 503 A1, published February 7, 2024. Title: MEDICAL USE OF CYCLIC PEPTIDE COMPOUNDS. Applicant: CHUGAI SEIYAKU KABUSHIKI KAISHA. The sequence listing filed with the application follows.

SEQUENCE LISTING (9 sequences)

SEQ ID NO: 1 - DNA, 615 bp, Artificial sequence
  HAT_Linker_Thrombin_Linker_hKras-G12D
atgaaagatcacctgattcacaatgtccataaagaagaacacgcccatgctcactcgtctggcagcctggtcccgcgtggttcgtcaggcgggagcaccgagtacaaactggtggttgtaggtgccgatggtgttggcaagagcgcgctgacgatccagttgattcaaaaccactttgtcgatgagtatgacccgacgatcgaggacagctaccgtaaacaagttgtgatcgatggcgagacttgcctgctggatattctggacacggctggccaagaagaatacagcgcgatgcgtgaccagtacatgcgcaccggtgagggtttcctgtgtgttttcgcaattaacaatacgaaatcctttgaggatattcatcactatcgtgaacagatcaagcgtgttaaagacagcgaagatgtcccgatggtgttggtgggcaataagtgcgatctgccgagccgcaccgtcgataccaaacaggcacaggacctggcgcgcagctatggtatcccgttcattgaaacctctgcgaaaacccgccaaggtgtcgacgacgccttttacaccctggtgcgtgagatccgtaagcataaggaaaagatgagcaaagacggc

SEQ ID NO: 2 - protein, 205 aa, Artificial sequence
  HAT_Linker_Thrombin_Linker_hKras-G12D
MKDHLIHNVHKEEHAHAHSSGSLVPRGSSGGSTEYKLVVVGADGVGKSALTIQLIQNHFVDEYDPTIEDSYRKQVVIDGETCLLDILDTAGQEEYSAMRDQYMRTGEGFLCVFAINNTKSFEDIHHYREQIKRVKDSEDVPMVLVGNKCDLPSRTVDTKQAQDLARSYGIPFIETSAKTRQGVDDAFYTLVREIRKHKEKMSKDG

SEQ ID NO: 3 - protein, 179 aa, Homo sapiens
GSSGGSTEYKLVVVGADGVGKSALTIQLIQNHFVDEYDPTIEDSYRKQVVIDGETCLLDILDTAGQEEYSAMRDQYMRTGEGFLCVFAINNTKSFEDIHHYREQIKRVKDSEDVPMVLVGNKCDLPSRTVDTKQAQDLARSYGIPFIETSAKTRQGVDDAFYTLVREIRKHKEKMSKDG

SEQ ID NO: 4 - protein, 17 aa, Artificial sequence
  HAT tag
KDHLIHNVHKEEHAHAH

SEQ ID NO: 5 - protein, 6 aa, Artificial sequence
  thrombin recognition sequence
LVPRGS

SEQ ID NO: 6 - protein, 189 aa, Homo sapiens [sequence omitted]

SEQ ID NO: 7 - protein, 189 aa, Homo sapiens
  source (1)..(189): hNRas wild type
MTEYKLVVVGAGGVGKSALTIQLIQNHFVDEYDPTIEDSYRKQVVIDGETCLLDILDTAGQEEYSAMRDQYMRTGEGFLCVFAINNSKSFADINLYREQIKRVKDSDDVPMVLVGNKCDLPTRTVDTKQAHELAKSYGIPFIETSAKTRQGVEDAFYTLVREIRQYRMKKLNSSDDGTQGCMGLPCVVM

SEQ ID NO: 8 - protein, 189 aa, Homo sapiens
  source (1)..(189): hHRas wild type
MTEYKLVVVGAGGVGKSALTIQLIQNHFVDEYDPTIEDSYRKQVVIDGETCLLDILDTAGQEEYSAMRDQYMRTGEGFLCVFAINNTKSFEDIHQYREQIKRVKDSDDVPMVLVGNKCDLAARTVESRQAQDLARSYGIPYIETSAKTRQGVEDAFYTLVREIRQHKLRKLNPPDESGPGCMSCKCVLS

SEQ ID NO: 9 - protein, 165 aa, Artificial sequence
  Ras consensus sequence
  misc_feature (12)..(12): Xaa = Gly, Asp, Cys, Ser, Val or Ala
  misc_feature (13)..(13): Xaa = Gly, Asp, Val or Arg
  misc_feature (61)..(61): Xaa = Gln, His, Lys or Leu
  misc_feature (87)..(87): Xaa = Thr or Ser
  misc_feature (91)..(91): Xaa = Glu or Ala
  misc_feature (94)..(94): Xaa = His or Asn
  misc_feature (95)..(95): Xaa = His, Leu or Gln
  misc_feature (107)..(107): Xaa = Glu or Asp
  misc_feature (121)..(121): Xaa = Pro or Ala
  misc_feature (122)..(122): Xaa = Ser, Thr or Ala
  misc_feature (126)..(126): Xaa = Asp or Glu
  misc_feature (127)..(127): Xaa = Thr or Ser
  misc_feature (128)..(128): Xaa = Lys or Arg
  misc_feature (131)..(131): Xaa = Gln or His
  misc_feature (132)..(132): Xaa = Asp or Glu
  misc_feature (135)..(135): Xaa = Arg or Lys
  misc_feature (141)..(141): Xaa = Phe or Tyr
  misc_feature (151)..(151): Xaa = Arg or Gly
MTEYKLVVVGAXXVGKSALTIQLIQNHFVDEYDPTIEDSYRKQVVIDGETCLLDILDTAGXEEYSAMRDQYMRTGEGFLCVFAINNXKSFXDIXXYREQIKRVKDSXDVPMVLVGNKCDLXXRTVXXXQAXXLAXSYGIPXIETSAKTRQXVEDAFYTLVREIRQ